European Patent Application EP 4 595 975 A1, published August 6, 2025. Title: FUSION PROTEIN FOR INDUCING IMMUNE RESPONSE AND TREATING CANCER. Applicant: TAIVITAL BIOPHARMACEUTICAL CO. LTD. Application EP. The sequence listing filed with the application follows.

SEQUENCE LISTING (10 sequences)

SEQ ID NO: 1 - protein, 252 aa, synthetic construct
AEEAFDLWNECAKACVLDLKDGVRSSRMSVDPAIADTNGQGVLHYSMVLEGGNDALKLAIDNALSITSDGLTIRLEGGVEPNKPVRYSYTRQARGSWSLNWLVPIGHEKPSNIKVFIHELNAGNQLSHMSPIYTIEMGDELLAKLARDATFFVRAHESNEMQPTLAISHAGVSVVMAQTQPRREKRWSEWASGKVLCLLDPLDGVYNYLAQQRCNLDDTWEGKIYRVLAGNPAKHDLDIKPTVISHRLHFPE

SEQ ID NO: 2 - protein, 112 aa, synthetic construct
GGSLAALTAHQACHLPLETFTRHRQPRGWEQLEQCGYPVQRLVALYLAARLSWNQVDQVIRNALASPGSGGDLGEAIREQPEQARLALTLAAAESERFVRQGTGNDEAGAAN

SEQ ID NO: 3 - protein, 40 aa, synthetic construct
ADVVSLTCPVAAGECAGPADSGDALLERNYPTGAEFLGDG

SEQ ID NO: 4 - protein, 10 aa, synthetic construct
PCCGCCGCGC

SEQ ID NO: 5 - protein, 70 aa, synthetic construct
PCCGCCGCGCPCCGCCGCGCPCCGCCGCGCPCCGCCGCGCPCCGCCGCGCPCCGCCGCGCPCCGCCGCGC

SEQ ID NO: 6 - protein, 4 aa, synthetic construct
KDEL

SEQ ID NO: 7 - protein, 4 aa, synthetic construct
RDEL

SEQ ID NO: 8 - protein, 5 aa, synthetic construct
REDLK

SEQ ID NO: 9 - protein, 503 aa, synthetic construct
MAEEAFDLWNECAKACVLDLKDGVRSSRMSVDPAIADTNGQGVLHYSMVLEGGNDALKLAIDNALSITSDGLTIRLEGGVEPNKPVRYSYTRQARGSWSLNWLVPIGHEKPSNIKVFIHELNAGNQLSHMSPIYTIEMGDELLAKLARDATFFVRAHESNEMQPTLAISHAGVSVVMAQTQPRREKRWSEWASGKVLCLLDPLDGVYNYLAQQRCNLDDTWEGKIYRVLAGNPAKHDLDIKPTVISHRLHFPEGGSLAALTAHQACHLPLETFTRHRQPRGWEQLEQCGYPVQRLVALYLAARLSWNQVDQVIRNALASPGSGGDLGEAIREQPEQARLALTLAAAESERFVRQGTGNDEAGAANADVVSLTCPVAAGECAGPADSGDALLERNYPTGAEFLGDGELGGGGSGSPCCGCCGCGCPCCGCCGCGCPCCGCCGCGCPCCGCCGCGCPCCGCCGCGCPCCGCCGCGCPCCGCCGCGCKLAAASGHHHHHHGREDLK

SEQ ID NO: 10 - protein, 209 aa, synthetic construct
GDVSFSTRGTQNWTVERLLQAHRQLEERGYVFVGYHGTFLEAAQSIVFGGVRARSQDLDAIWRGFYIAGDPALAYGYAQDQEPDARGRIRNGALLRVYVPRSSLPGFYRTSLTLAAPEAAGEVERLIGHPLPLRLDAITGPEEEGGRLETILGWPLAERTVVIPSAIPTDPRNVGGDLDPSSIPDKEQAISALPDYASQPGKPPREDLK